European Patent Application EP 4 467 152 A1, published November 27, 2024. Title: Peptides for use in the prevention and/or treatment of radiodermatitis. Applicant: Alodia Farmacéutica S.L.U. Application ES. The sequence listing filed with the application follows.

SEQUENCE LISTING (33 sequences)

SEQ ID NO: 1 - protein, 11 aa, Homo sapiens
GFINLDKPSNP

SEQ ID NO: 2 - protein, 19 aa, Homo sapiens
GFINLDKPSNPSSHEVVAW

SEQ ID NO: 3 - protein, 25 aa, Homo sapiens
GFINLDKPSNPSSHEVVAWIRRILR

SEQ ID NO: 4 - protein, 55 aa, Homo sapiens
GFINLDKPSNPSSHEVVAWIRRILRVEKTGHSGTLDPKVTGCLIVCIERATRLVK

SEQ ID NO: 5 - protein, 17 aa, Homo sapiens
GFINLDKPSNPSSHEVV

SEQ ID NO: 6 - protein, 18 aa, Homo sapiens
GFINLDKPSNPSSHEVVA

SEQ ID NO: 7 - protein, 4 aa, synthetic construct
KRKR

SEQ ID NO: 8 - protein, 8 aa, synthetic construct
KKEKKKSK

SEQ ID NO: 9 - protein, 15 aa, synthetic construct
GFINLDKPSNPKRKR

SEQ ID NO: 10 - protein, 59 aa, synthetic construct
GFINLDKPSNPSSHEVVAWIRRILRVEKTGHSGTLDPKVTGCLIVCIERATRLVKKRKR

SEQ ID NO: 11 - protein, 63 aa, synthetic construct
GFINLDKPSNPSSHEVVAWIRRILRVEKTGHSGTLDPKVTGCLIVCIERATRLVKKKEKKKSK

SEQ ID NO: 12 - protein, 59 aa, unidentified
KRKRGFINLDKPSNPSSHEVVAWIRRILRVEKTGHSGTLDPKVTGCLIVCIERATRLVK

SEQ ID NO: 13 - protein, 62 aa, synthetic construct
KKEKKKSKGFINLDKPSNPSSHEWAWIRRILRVEKTGHSGTLDPKVTGCLIVCIERATRLVK

SEQ ID NO: 14 - protein, 15 aa, synthetic construct
KRKRGFINLDKPSNP

SEQ ID NO: 15 - protein, 19 aa, synthetic construct
GFINLDKPSNPKKEKKKSK

SEQ ID NO: 16 - protein, 19 aa, synthetic construct
KKEKKKSKGFINLDKPSNP

SEQ ID NO: 17 - DNA, 33 bp, Homo sapiens
  source 1..33: mol_type = genomic DNA
ggtttcattaatcttgacaagccctctaacccc

SEQ ID NO: 18 - DNA, 57 bp, Homo sapiens
  source 1..57: mol_type = genomic DNA
ggtttcattaatcttgacaagccctctaacccctcttcccatgaggtggtagcctgg

SEQ ID NO: 19 - DNA, 75 bp, Homo sapiens
  source 1..75: mol_type = genomic DNA
ggtttcattaatcttgacaagccctctaacccctcttcccatgaggtggtagcctggattcgacggatacttcgg

SEQ ID NO: 20 - DNA, 165 bp, Homo sapiens
  source 1..165: mol_type = genomic DNA
ggtttcattaatcttgacaagccctctaacccctcttcccatgaggtggtagcctggattcgacggatacttcgggtggagaagacagggcacagtggtactctggatcccaaggtgactggttgtttaatcgtgtgcatagaacgagccactcgcttggtgaag

SEQ ID NO: 21 - DNA, 51 bp, Homo sapiens
  source 1..51: mol_type = genomic DNA
ggtttcattaatcttgacaagccctctaacccctcttcccatgaggtggta

SEQ ID NO: 22 - DNA, 54 bp, Homo sapiens
  source 1..54: mol_type = genomic DNA
ggtttcattaatcttgacaagccctctaacccctcttcccatgaggtggtagcc

SEQ ID NO: 23 - protein, 9 aa, Human immunodeficiency virus 1
  source 1..9: organism (original language) = Virus de la inmunodeficiencia humana 1
RKKRRQRRR

SEQ ID NO: 24 - protein, 11 aa, Human immunodeficiency virus 1
  source 1..11: organism (original language) = Virus de la inmunodeficiencia humana 1
YGRKKRRQRRR

SEQ ID NO: 25 - protein, 15 aa, Human immunodeficiency virus 1
  source 1..15: organism (original language) = Virus de la inmunodeficiencia humana 1
CGISYGRKKRRQRRR

SEQ ID NO: 26 - protein, 16 aa, Drosophila melanogaster
RQIKIWFQNRRMKWKK

SEQ ID NO: 27 - protein, 19 aa, Homo sapiens
KFVRSRRPRTASCALAFVN

SEQ ID NO: 28 - protein, 8 aa, Homo sapiens
SCALAFVN

SEQ ID NO: 29 - protein, 11 aa, synthetic construct
YTDIEMNRLGK

SEQ ID NO: 30 - protein, 6 aa, synthetic construct
AHGHRP

SEQ ID NO: 31 - protein, 14 aa, synthetic construct
PIHDHDHPHLVIHS

SEQ ID NO: 32 - protein, 7 aa, synthetic construct
PKKKRKV

SEQ ID NO: 33 - protein, 19 aa, synthetic construct
MDWTWRVFCLLAVTPGAHP